European Patent Specification EP 3 494 123 B1, published September 25, 2024. Title: RNAi Agents for Hepatitis B Virus Infection. Applicant: ARROWHEAD PHARMACEUTICALS, INC. Zhen Li Rui Zhu Christine I. Wooddell Bruce D. Given Tao Pei David L. Lewis Lauren J. Almeida David B. Rozema Darren H. Wakefield. The sequence listing filed with the application follows.

SEQUENCE LISTING (334 sequences)

SEQ ID NO: 1 - DNA, 3221 bp, Artificial sequence
  Hepatitis B virus (subtype ADW2), genotype A, complete gene (AM282986.1)
ttccactgccttccaccaagctctgcaggatcccaaagtcaggggtctgtattttcctgctggtggctccagttcaggaacagtaaaccctgctccgaatattgcctctcacatctcgtcaatctccgcgaggactggggaccctgtgacgaatatggagaacatcacatcaggattcctaggacccctgctcgtgttacaggcggggtttttcttgttgacaagaatcctcacaataccgcagagtctagactcgtggtggacttctctcaattttctagggggatcacccgtgtgtcttggccaaaattcgcagtccccaacctccaatcactcaccaacctcctgtcctccaatttgtcctggttatcgctggatgtgtctgcggcgttttatcatattcctcttcatcctgctgctatgcctcatcttcttgttggttcttctggattatcaaggtatgttgcccgtttgtcctctaattccaggaacaacaacaaccagtacgggaccatgcaaaacctgcacgactcctgctcaaggcaactctatgtttccctcatgttgctgtacaaaaccttcggatggaaattgcacctgtattcccatcccatcgtcttgggctttcgcaaaatacctatgggagtgggcctcagtccgtttctcttggctcagtttactagtgccatttgttcagtggttcgtagggctttcccccactgtttggctttcagctatatggatgatgtggtattgggggccaagtctgtacagcatcgtgagtccctttataccgctgttaccaattttcttttgtctctgggtatacatttaaaccctaacaaaacaaaaagatggggttattccctaaacttcatgggttacataattggaagttggggaacgttgccacaggatcatattgtacaaaagatcaaacactgttttagaaaacttcctgttaacaggcctattgattggaaagtatgtcaaagaattgtgggtcttttgggctttgctgctccatttacacaatgtggatatcctgccttaatgcctttgtatgcctgtatacaagctaaacaggctttcactttctcgccaacttacaaggcctttctaagtaaacagtacatgaacctttaccccgttgctcggcaacggcctggtctgtgccaagtgtttgctgacgcaacccccactggctggggcttggccataggccatcagcgcatgcgtggaacctttgtggctcctctgccgatccatactgcggaactcctagccgcttgttttgctcgcagccggtctggggcaaagctcatcggaactgacaattctgtcgtcctctcgcggaaatatacatcgtttccatggctgctaggttgtactgccaactggatccttcgcgggacgtcctttgtttacgtcccgtcggcgctgaatcccgcggacgacccctctcggggccgcttgggactctctcgtccccttctccgtctgccgttccagccgaccacggggcgcacctctctttacgcggtctccccgtctgtgccttctcatctgccggtccgtgtgcacttcgcttcacctctgcacgttgcatggagaccaccgtgaacgcccatcagatcctgcccaaggtcttacataagaggactcttggactcccagcaatgtcaacgaccgaccttgaggcctacttcaaagactgtgtgtttaaggactgggaggagctgggggaggagattaggttaaaggtctttgtattaggaggctgtaggcataaattggtctgcgcaccagcaccatgcaactttttcacctctgcctaatcatctcttgtacatgtcccactgttcaagcctccaagctgtgccttgggtggctttggggcatggacattgacccttataaagaatttggagctactgtggagttactctcgtttttgccttctgacttttttccttccgtcagagatctcctagacaccgcctcagctctgtatcgggaagccttagagtctcctgagcattgctcacctcaccatactgcactcaggcaagcaattctctgctggggggaattgatgactctagctacctgggtgggtaataatttggaagatccagcatccagggatctagtagtcaattatgttaatactaacatgggtttaaagatcaggcaactattgtggtttcatatatcttgccttacttttggaagagagactgtacttgaatatttggtctctttcggagtgtggattcgcactcctccagcctatagaccaccaaatgcccctatcttatcaacacttccggaaactactgttgttagacgacgggaccgaggcaggtcccctagaagaagaactccctcgcctcgcagacgcagatctcaatcgccgcgtcgcagaagatctcaatctcgggaatctcaatgttagtattccttggactcataaggtgggaaactttactgggctttattcctctacagtacctatctttaatcctgaatggcaaactccttcctttcctaagattcatttacaagaggacattattaataggtgtcaacaatttgtgggccctctcactgtaaatgaaaagagaagattgaaattaattatgcctgctagattctatcctacccacactaaatatttgcccttagacaaaggaattaaaccttattatccagatcaggtagttaatcattacttcaaaaccagacattatttacatactctttggaaggctggtattctatataagagggaaaccacacgtagcgcatcattttgcgggtcaccatattcttgggaacaagagctacagcatgggaggttggtcatcgaaacctcgcaaaggcatggggacgaatctttctgttcccaaccctctgggattctttcccgatcatcagttggaccctgcattcggagccaactcaaacaatccagattgggacttcaaccccatcaaggaccactggccagcagccaaccaggtaggagtgggagcattcgggccagggttcacccctccacacggcggtgttttggggtggagccctcaggctcagggcatattgaccacagtgtcaacaattcctcctcctgcctccaccaatcggcagtcaggaaggcagcctactcccatctctccacctctaagagacagtcatcctcaggccatgcagtggaa

SEQ ID NO: 2 - DNA, 19 bp, Artificial sequence
  HBV cDNA target sequence
gtggtggacttctctcaat

SEQ ID NO: 3 - DNA, 19 bp, Artificial sequence
  HBV cDNA target sequence
tggtggacttctctcaatt

SEQ ID NO: 4 - DNA, 19 bp, Artificial sequence
  HBV cDNA target sequence
ggacttctctcaattttct

SEQ ID NO: 5 - DNA, 19 bp, Artificial sequence
  HBV cDNA target sequence
gctgtaggcataaattggt

SEQ ID NO: 6 - DNA, 19 bp, Artificial sequence
  HBV cDNA target sequence
ctgtaggcataaattggtc

SEQ ID NO: 7 - RNA, 19 nt, Artificial sequence
  HBV RNAi agent antisense strand core stretch sequence
auugagagaaguccaccac

SEQ ID NO: 8 - RNA, 19 nt, Artificial sequence
  HBV RNAi agent antisense strand core stretch sequence
uuugagagaaguccaccac

SEQ ID NO: 9 - RNA, 19 nt, Artificial sequence
  HBV RNAi agent antisense strand core stretch sequence
  modified_base 19: n = any nucleotide
auugagagaaguccaccan

SEQ ID NO: 10 - RNA, 19 nt, Artificial sequence
  HBV RNAi agent antisense strand core stretch sequence
  modified_base 19: n = any nucleotide
uuugagagaaguccaccan

SEQ ID NO: 11 - RNA, 19 nt, Artificial sequence
  HBV RNAi agent antisense strand core stretch sequence
  modified_base 1, 19: n = any nucleotide
nuugagagaaguccaccan

SEQ ID NO: 12 - RNA, 19 nt, Artificial sequence
  HBV RNAi agent antisense strand core stretch sequence
aauugagagaaguccacca

SEQ ID NO: 13 - RNA, 19 nt, Artificial sequence
  HBV RNAi agent antisense strand core stretch sequence
uauugagagaaguccacca

SEQ ID NO: 14 - RNA, 19 nt, Artificial sequence
  HBV RNAi agent antisense strand core stretch sequence
  modified_base 19: n = any nucleotide
aauugagagaaguccaccn

SEQ ID NO: 15 - RNA, 19 nt, Artificial sequence
  HBV RNAi agent antisense strand core stretch sequence
  modified_base 19: n = any nucleotide
uauugagagaaguccaccn

SEQ ID NO: 16 - RNA, 19 nt, Artificial sequence
  HBV RNAi agent antisense strand core stretch sequence
  modified_base 1, 19: n = any nucleotide
nauugagagaaguccaccn

SEQ ID NO: 17 - RNA, 19 nt, Artificial sequence
  HBV RNAi agent antisense strand core stretch sequence
agaaaauugagagaagucc

SEQ ID NO: 18 - RNA, 19 nt, Artificial sequence
  HBV RNAi agent antisense strand core stretch sequence
ugaaaauugagagaagucc

SEQ ID NO: 19 - RNA, 19 nt, Artificial sequence
  HBV RNAi agent antisense strand core stretch sequence
  modified_base 19: n = any nucleotide
agaaaauugagagaagucn

SEQ ID NO: 20 - RNA, 19 nt, Artificial sequence
  HBV RNAi agent antisense strand core stretch sequence
  modified_base 19: n = any nucleotide
ugaaaauugagagaagucn

SEQ ID NO: 21 - RNA, 19 nt, Artificial sequence
  HBV RNAi agent antisense strand core stretch sequence
  modified_base 1, 19: n = any nucleotide
ngaaaauugagagaagucn

SEQ ID NO: 22 - RNA, 19 nt, Artificial sequence
  HBV RNAi agent antisense strand core stretch sequence
accaauuuaugccuacagc

SEQ ID NO: 23 - RNA, 19 nt, Artificial sequence
  HBV RNAi agent antisense strand core stretch sequence
uccaauuuaugccuacagc

SEQ ID NO: 24 - RNA, 19 nt, Artificial sequence
  HBV RNAi agent antisense strand core stretch sequence
  modified_base 19: n = any nucleotide
accaauuuaugccuacagn

SEQ ID NO: 25 - RNA, 19 nt, Artificial sequence
  HBV RNAi agent antisense strand core stretch sequence
  modified_base 19: n = any nucleotide
uccaauuuaugccuacagn

SEQ ID NO: 26 - RNA, 19 nt, Artificial sequence
  HBV RNAi agent antisense strand core stretch sequence
  modified_base 1,19: n = any nucleotide
nccaauuuaugccuacagn

SEQ ID NO: 27 - RNA, 19 nt, Artificial sequence
  HBV RNAi agent antisense strand core stretch sequence
gaccaauuuaugccuacag

SEQ ID NO: 28 - RNA, 19 nt, Artificial sequence
  HBV RNAi agent antisense strand core stretch sequence
aaccaauuuaugccuacag

SEQ ID NO: 29 - RNA, 19 nt, Artificial sequence
  HBV RNAi agent antisense strand core stretch sequence
uaccaauuuaugccuacag

SEQ ID NO: 30 - RNA, 19 nt, Artificial sequence
  HBV RNAi agent antisense strand core stretch sequence
  modified_base 19: n = any nucleotide
gaccaauuuaugccuacan

SEQ ID NO: 31 - RNA, 19 nt, Artificial sequence
  HBV RNAi agent antisense strand core stretch sequence
  modified_base 19: n = any nucleotide
aaccaauuuaugccuacan

SEQ ID NO: 32 - RNA, 19 nt, Artificial sequence
  HBV RNAi agent antisense strand core stretch sequence
  modified_base 19: n = any nucleotide
uaccaauuuaugccuacan

SEQ ID NO: 33 - RNA, 19 nt, Artificial sequence
  HBV RNAi agent antisense strand core stretch sequence
  modified_base 1, 19: n = any nucleotide
naccaauuuaugccuacan

SEQ ID NO: 34 - DNA, 19 bp, Artificial sequence
  HBV RNAi agent sense strand core stretch sequence
gugguggacuucucucaau

SEQ ID NO: 35 - RNA, 19 nt, Artificial sequence
  HBV RNAi agent sense strand core stretch sequence
gugguggacuucucucaaa

SEQ ID NO: 36 - RNA, 19 nt, Artificial sequence
  HBV RNAi agent sense strand core stretch sequence
  modified_base 1: n = any nucleotide
nugguggacuucucucaau

SEQ ID NO: 37 - RNA, 19 nt, Artificial sequence
  HBV RNAi agent sense strand core stretch sequence
  modified_base 1: n = any nucleotide
nugguggacuucucucaaa

SEQ ID NO: 38 - RNA, 19 nt, Artificial sequence
  HBV RNAi agent sense strand core stretch sequence
  modified_base 1, 19: n = any nucleotide
nugguggacuucucucaan

SEQ ID NO: 39 - RNA, 19 nt, Artificial sequence
  HBV RNAi agent sense strand core stretch sequence
ugguggacuucucucaauu

SEQ ID NO: 40 - RNA, 19 nt, Artificial sequence
  HBV RNAi agent sense strand core stretch sequence
ugguggacuucucucaaua

SEQ ID NO: 41 - RNA, 19 nt, Artificial sequence
  HBV RNAi agent sense strand core stretch sequence
  modified_base 1: n = any nucleotide
ngguggacuucucucaauu

SEQ ID NO: 42 - RNA, 19 nt, Artificial sequence
  HBV RNAi agent sense strand core stretch sequence
  modified_base 1: n = any nucleotide
ngguggacuucucucaaua

SEQ ID NO: 43 - RNA, 19 nt, Artificial sequence
  HBV RNAi agent sense strand core stretch sequence
  modified_base 1, 19: n = any nucleotide
ngguggacuucucucaaun

SEQ ID NO: 44 - RNA, 19 nt, Artificial sequence
  HBV RNAi agent sense strand core stretch sequence
ggacuucucucaauuuucu

SEQ ID NO: 45 - RNA, 19 nt, Artificial sequence
  HBV RNAi agent sense strand core stretch sequence
ggacuucucucaauuuuca

SEQ ID NO: 46 - RNA, 19 nt, Artificial sequence
  HBV RNAi agent sense strand core stretch sequence
  modified_base 1: n = any nucleotide
ngacuucucucaauuuucu

SEQ ID NO: 47 - RNA, 19 nt, Artificial sequence
  HBV RNAi agent sense strand core stretch sequence
  modified_base 1: n = any nucleotide
ngacuucucucaauuuuca

SEQ ID NO: 48 - RNA, 19 nt, Artificial sequence
  HBV RNAi agent sense strand core stretch sequence
  modified_base 1, 19: n = any nucleotide
ngacuucucucaauuuucn

SEQ ID NO: 49 - RNA, 19 nt, Artificial sequence
  HBV RNAi agent sense strand core stretch sequence
gcuguaggcauaaauuggu

SEQ ID NO: 50 - RNA, 19 nt, Artificial sequence
  HBV RNAi agent sense strand core stretch sequence
gcuguaggcauaaauugga

SEQ ID NO: 51 - RNA, 19 nt, Artificial sequence
  HBV RNAi agent sense strand core stretch sequence
  modified_base 1: n = any nucleotide
ncuguaggcauaaauuggu

SEQ ID NO: 52 - RNA, 19 nt, Artificial sequence
  HBV RNAi agent sense strand core stretch sequence
  modified_base 1: n = any nucleotide
ncuguaggcauaaauugga

SEQ ID NO: 53 - RNA, 19 nt, Artificial sequence
  HBV RNAi agent sense strand core stretch sequence
  modified_base 1, 19: n = any nucleotide
ncuguaggcauaaauuggn

SEQ ID NO: 54 - RNA, 19 nt, Artificial sequence
  HBV RNAi agent sense strand core stretch sequence
cuguaggcauaaauugguc

SEQ ID NO: 55 - RNA, 19 nt, Artificial sequence
  HBV RNAi agent sense strand core stretch sequence
cuguaggcauaaauugguu

SEQ ID NO: 56 - RNA, 19 nt, Artificial sequence
  HBV RNAi agent sense strand core stretch sequence
cuguaggcauaaauuggua

SEQ ID NO: 57 - RNA, 19 nt, Artificial sequence
  HBV RNAi agent sense strand core stretch sequence
  modified_base 1: n = any nucleotide
nuguaggcauaaauugguc

SEQ ID NO: 58 - RNA, 19 nt, Artificial sequence
  HBV RNAi agent sense strand core stretch sequence
  modified_base 1: n = any nucleotide
nuguaggcauaaauugguu

SEQ ID NO: 59 - RNA, 19 nt, Artificial sequence
  HBV RNAi agent sense strand core stretch sequence
  modified_base 1: n = any nucleotide
nuguaggcauaaauuggua

SEQ ID NO: 60 - RNA, 19 nt, Artificial sequence
  HBV RNAi agent sense strand core stretch sequence
  modified_base 1, 19: n = any nucleotide
nuguaggcauaaauuggun

SEQ ID NO: 61 - RNA, 26 nt, Artificial sequence
  HBV RNAi Agent antisense strand modified sequence
uaccaauuuaugccuacaggccuuau

SEQ ID NO: 62 - RNA, 23 nt, Artificial sequence
  HBV RNAi Agent antisense strand modified sequence
uaccaauuuaugccuacaggccu

SEQ ID NO: 63 - RNA, 23 nt, Artificial sequence
  HBV RNAi Agent antisense strand modified sequence
uaccaauuuaugccuacaggccu

SEQ ID NO: 64 - RNA, 21 nt, Artificial sequence
  HBV RNAi Agent antisense strand modified sequence
uaccaauuuaugccuacaggc

SEQ ID NO: 65 - RNA, 21 nt, Artificial sequence
  HBV RNAi Agent antisense strand modified sequence
ugugaagcgaagugcacacuu

SEQ ID NO: 66 - RNA, 26 nt, Artificial sequence
  HBV RNAi Agent antisense strand modified sequence
uaccaauuuaugccuacagccuccgc

SEQ ID NO: 67 - RNA, 26 nt, Artificial sequence
  HBV RNAi Agent antisense strand modified sequence
uaccaauuuaugccuacagccuccgc

SEQ ID NO: 68 - RNA, 21 nt, Artificial sequence
  HBV RNAi Agent antisense strand modified sequence
uaccaauuuaugccuacaguu

SEQ ID NO: 69 - RNA, 21 nt, Artificial sequence
  HBV RNAi Agent antisense strand modified sequence
uaccaauuuaugccuacaggc

SEQ ID NO: 70 - RNA, 21 nt, Artificial sequence
  HBV RNAi Agent antisense strand modified sequence
uaccaauuuaugccuacaggc

SEQ ID NO: 71 - RNA, 21 nt, Artificial sequence
  HBV RNAi Agent antisense strand modified sequence
uaccaauuuaugccuacaguu

SEQ ID NO: 72 - RNA, 21 nt, Artificial sequence
  HBV RNAi Agent antisense strand modified sequence
auugagagaaguccaccacga

SEQ ID NO: 73 - RNA, 21 nt, Artificial sequence
  HBV RNAi Agent antisense strand modified sequence
auugagagaaguccaccacga

SEQ ID NO: 74 - RNA, 21 nt, Artificial sequence
  HBV RNAi Agent antisense strand modified sequence
auugagagaaguccaccacuu

SEQ ID NO: 75 - RNA, 21 nt, Artificial sequence
  HBV RNAi Agent antisense strand modified sequence
uuugagagaaguccaccacga

SEQ ID NO: 76 - RNA, 21 nt, Artificial sequence
  HBV RNAi Agent antisense strand modified sequence
aauugagagaaguccaccacg

SEQ ID NO: 77 - RNA, 21 nt, Artificial sequence
  HBV RNAi Agent antisense strand modified sequence
aauugagagaaguccaccacg

SEQ ID NO: 78 - RNA, 21 nt, Artificial sequence
  HBV RNAi Agent antisense strand modified sequence
aauugagagaaguccaccauu

SEQ ID NO: 79 - RNA, 21 nt, Artificial sequence
  HBV RNAi Agent antisense strand modified sequence
uauugagagaaguccaccacg

SEQ ID NO: 80 - RNA, 21 nt, Artificial sequence
  HBV RNAi Agent antisense strand modified sequence
uaccaauuuaugccuacaggu

SEQ ID NO: 81 - RNA, 21 nt, Artificial sequence
  HBV RNAi Agent antisense strand modified sequence
uaccaauuuaugccuacaguu

SEQ ID NO: 82 - RNA, 21 nt, Artificial sequence
  HBV RNAi Agent antisense strand modified sequence
uaccaauuuaugccuacagcc

SEQ ID NO: 83 - RNA, 23 nt, Artificial sequence
  HBV RNAi Agent antisense strand modified sequence
uaccaauuuaugccuacagccuu

SEQ ID NO: 84 - RNA, 23 nt, Artificial sequence
  HBV RNAi Agent antisense strand modified sequence
uaccaauuuaugccuacagccuc

SEQ ID NO: 85 - RNA, 21 nt, Artificial sequence
  HBV RNAi Agent antisense strand modified sequence
uaccaauuuaugccuacagcc

SEQ ID NO: 86 - RNA, 23 nt, Artificial sequence
  HBV RNAi Agent antisense strand modified sequence
uaccaauuuaugccuacagccuu

SEQ ID NO: 87 - RNA, 23 nt, Artificial sequence
  HBV RNAi Agent antisense strand modified sequence
uaccaauuuaugccuacagccuc

SEQ ID NO: 88 - RNA, 21 nt, Artificial sequence
  HBV RNAi Agent antisense strand modified sequence
auugagagaaguccaccacuu

SEQ ID NO: 89 - RNA, 21 nt, Artificial sequence
  HBV RNAi Agent antisense strand modified sequence
uuugagagaaguccaccacuu

SEQ ID NO: 90 - RNA, 23 nt, Artificial sequence
  HBV RNAi Agent antisense strand modified sequence
auugagagaaguccaccacgguu

SEQ ID NO: 91 - RNA, 23 nt, Artificial sequence
  HBV RNAi Agent antisense strand modified sequence
auugagagaaguccaccacgguu

SEQ ID NO: 92 - RNA, 23 nt, Artificial sequence
  HBV RNAi Agent antisense strand modified sequence
auugagagaaguccaccacgagu

SEQ ID NO: 93 - RNA, 21 nt, Artificial sequence
  HBV RNAi Agent antisense strand modified sequence
uauugagagaaguccaccacg

SEQ ID NO: 94 - RNA, 21 nt, Artificial sequence
  HBV RNAi Agent antisense strand modified sequence
uauugagagaaguccaccacg

SEQ ID NO: 95 - RNA, 23 nt, Artificial sequence
  HBV RNAi Agent antisense strand modified sequence
uauugagagaaguccaccacguu

SEQ ID NO: 96 - RNA, 23 nt, Artificial sequence
  HBV RNAi Agent antisense strand modified sequence
uauugagagaaguccaccacgag

SEQ ID NO: 97 - RNA, 23 nt, Artificial sequence
  HBV RNAi Agent antisense strand modified sequence
uauugagagaaguccaccacgag

SEQ ID NO: 98 - RNA, 22 nt, Artificial sequence
  HBV RNAi Agent antisense strand modified sequence
uauugagagaaguccaccacga

SEQ ID NO: 99 - RNA, 22 nt, Artificial sequence
  HBV RNAi Agent antisense strand modified sequence
uauugagagaaguccaccacga

SEQ ID NO: 100 - RNA, 21 nt, Artificial sequence
  HBV RNAi Agent antisense strand modified sequence
agaaaauugagagaaguccac

SEQ ID NO: 101 - RNA, 21 nt, Artificial sequence
  HBV RNAi Agent antisense strand modified sequence
uaccaauuuaugccuacaguu

SEQ ID NO: 102 - RNA, 21 nt, Artificial sequence
  HBV RNAi Agent antisense strand modified sequence
uaccaauuuaugccuacagcc

SEQ ID NO: 103 - RNA, 22 nt, Artificial sequence
  HBV RNAi Agent antisense strand modified sequence
uaccaauuuaugccuacagcuu

SEQ ID NO: 104 - RNA, 22 nt, Artificial sequence
  HBV RNAi Agent antisense strand modified sequence
uaccaauuuaugccuacagccu

SEQ ID NO: 105 - RNA, 23 nt, Artificial sequence
  HBV RNAi Agent antisense strand modified sequence
uaccaauuuaugccuacagccuu

SEQ ID NO: 106 - RNA, 23 nt, Artificial sequence
  HBV RNAi Agent antisense strand modified sequence
uaccaauuuaugccuacagccuc

SEQ ID NO: 107 - RNA, 21 nt, Artificial sequence
  HBV RNAi Agent antisense strand modified sequence
uaccaauuuaugccuacaguu

SEQ ID NO: 108 - RNA, 21 nt, Artificial sequence
  HBV RNAi Agent antisense strand modified sequence
uauugagagaaguccaccacg

SEQ ID NO: 109 - RNA, 21 nt, Artificial sequence
  HBV RNAi Agent antisense strand modified sequence
uauugagagaaguccaccauu

SEQ ID NO: 110 - RNA, 21 nt, Artificial sequence
  HBV RNAi Agent antisense strand modified sequence
uauugagagaaguccaccacg

SEQ ID NO: 111 - RNA, 22 nt, Artificial sequence
  HBV RNAi Agent antisense strand modified sequence
uauugagagaaguccaccacuu

SEQ ID NO: 112 - RNA, 22 nt, Artificial sequence
  HBV RNAi Agent antisense strand modified sequence
uauugagagaaguccaccacga

SEQ ID NO: 113 - RNA, 21 nt, Artificial sequence
  HBV RNAi Agent antisense strand modified sequence
uauugagagaaguccaccacg

SEQ ID NO: 114 - RNA, 21 nt, Artificial sequence
  HBV RNAi Agent antisense strand modified sequence
uuugagagaaguccaccacuu

SEQ ID NO: 115 - RNA, 21 nt, Artificial sequence
  HBV RNAi Agent antisense strand modified sequence
uuugagagaaguccaccacga

SEQ ID NO: 116 - RNA, 22 nt, Artificial sequence
  HBV RNAi Agent antisense strand modified sequence
uuugagagaaguccaccacguu

SEQ ID NO: 117 - RNA, 22 nt, Artificial sequence
  HBV RNAi Agent antisense strand modified sequence
uuugagagaaguccaccacgag

SEQ ID NO: 118 - RNA, 21 nt, Artificial sequence
  HBV RNAi Agent antisense strand modified sequence
uuugagagaaguccaccacuu

SEQ ID NO: 119 - RNA, 22 nt, Artificial sequence
  HBV RNAi Agent antisense strand modified sequence
uauugagagaaguccaccacuu

SEQ ID NO: 120 - RNA, 22 nt, Artificial sequence
  HBV RNAi Agent antisense strand modified sequence
uauugagagaaguccaccacuu

SEQ ID NO: 121 - RNA, 23 nt, Artificial sequence
  HBV RNAi Agent antisense strand modified sequence
uauugagagaaguccaccacguu

SEQ ID NO: 122 - RNA, 22 nt, Artificial sequence
  HBV RNAi Agent antisense strand modified sequence
uauugagagaaguccaccacuu

SEQ ID NO: 123 - RNA, 23 nt, Artificial sequence
  HBV RNAi Agent antisense strand modified sequence
uauugagagaaguccaccacgag

SEQ ID NO: 124 - RNA, 22 nt, Artificial sequence
  HBV RNAi Agent antisense strand modified sequence
uauugagagaaguccaccacuu

SEQ ID NO: 125 - RNA, 21 nt, Artificial sequence
  HBV RNAi Agent antisense strand modified sequence
agaaaauugagagaaguccuu

SEQ ID NO: 126 - RNA, 21 nt, Artificial sequence
  HBV RNAi Agent antisense strand modified sequence
agaaaauugagagaaguccac

SEQ ID NO: 127 - RNA, 23 nt, Artificial sequence
  HBV RNAi Agent antisense strand modified sequence
agaaaauugagagaaguccacuu

SEQ ID NO: 128 - RNA, 22 nt, Artificial sequence
  HBV RNAi Agent antisense strand modified sequence
agaaaauugagagaaguccacc

SEQ ID NO: 129 - RNA, 21 nt, Artificial sequence
  HBV RNAi Agent antisense strand modified sequence
ugaaaauugagagaaguccuu

SEQ ID NO: 130 - RNA, 21 nt, Artificial sequence
  HBV RNAi Agent antisense strand modified sequence
ugaaaauugagagaaguccac

SEQ ID NO: 131 - RNA, 21 nt, Artificial sequence
  HBV RNAi Agent antisense strand modified sequence
accaauuuaugccuacagcuu

SEQ ID NO: 132 - RNA, 22 nt, Artificial sequence
  HBV RNAi Agent antisense strand modified sequence
accaauuuaugccuacagccuu

SEQ ID NO: 133 - RNA, 22 nt, Artificial sequence
  HBV RNAi Agent antisense strand modified sequence
accaauuuaugccuacagccuc

SEQ ID NO: 134 - RNA, 21 nt, Artificial sequence
  HBV RNAi Agent antisense strand modified sequence
uccaauuuaugccuacagcuu

SEQ ID NO: 135 - RNA, 22 nt, Artificial sequence
  HBV RNAi Agent antisense strand modified sequence
uccaauuuaugccuacagccuu

SEQ ID NO: 136 - RNA, 21 nt, Artificial sequence
  HBV RNAi Agent antisense strand modified sequence
uaccaauuuaugccuacagcc

SEQ ID NO: 137 - RNA, 21 nt, Artificial sequence
  HBV RNAi Agent antisense strand modified sequence
uaccaauuuaugccuacagcc

SEQ ID NO: 138 - RNA, 21 nt, Artificial sequence
  HBV RNAi Agent antisense strand modified sequence
uaccaauuuaugccuacagcc

SEQ ID NO: 139 - RNA, 21 nt, Artificial sequence
  HBV RNAi Agent antisense strand modified sequence
uaccaauuuaugccuacagcu

SEQ ID NO: 140 - RNA, 21 nt, Artificial sequence
  HBV RNAi Agent antisense strand modified sequence
uaccaauuuaugccuacagcg

SEQ ID NO: 141 - RNA, 21 nt, Artificial sequence
  HBV RNAi Agent antisense strand modified sequence
aaccaauuuaugccuacagcc

SEQ ID NO: 142 - RNA, 21 nt, Artificial sequence
  HBV RNAi Agent antisense strand modified sequence
uaccaauuuaugccuacaguu

SEQ ID NO: 143 - RNA, 21 nt, Artificial sequence
  HBV RNAi Agent antisense strand modified sequence
uaccaauuuaugccuacagcc

SEQ ID NO: 144 - RNA, 21 nt, Artificial sequence
  HBV RNAi Agent antisense strand modified sequence
accaauuuaugccuacagccu

SEQ ID NO: 145 - RNA, 21 nt, Artificial sequence
  HBV RNAi Agent antisense strand modified sequence
uccaauuuaugccuacagccu

SEQ ID NO: 146 - RNA, 21 nt, Artificial sequence
  HBV RNAi Agent antisense strand modified sequence
accaauuuaugccuacagccg

SEQ ID NO: 147 - RNA, 21 nt, Artificial sequence
  HBV RNAi Agent antisense strand modified sequence
uccaauuuaugccuacagccg

SEQ ID NO: 148 - RNA, 21 nt, Artificial sequence
  HBV RNAi Agent antisense strand modified sequence
uaccaauuuaugccuacaggg

SEQ ID NO: 149 - RNA, 26 nt, Artificial sequence
  HBV RNAi Agent antisense strand unmodified sequence
uaccaauuuaugccuacaggccuuau

SEQ ID NO: 150 - RNA, 23 nt, Artificial sequence
  HBV RNAi Agent antisense strand unmodified sequence
uaccaauuuaugccuacaggccu

SEQ ID NO: 151 - RNA, 21 nt, Artificial sequence
  HBV RNAi Agent antisense strand unmodified sequence
uaccaauuuaugccuacaggc

SEQ ID NO: 152 - RNA, 21 nt, Artificial sequence
  HBV RNAi Agent antisense strand unmodified sequence
ugugaagcgaagugcacacuu

SEQ ID NO: 153 - RNA, 26 nt, Artificial sequence
  HBV RNAi Agent antisense strand unmodified sequence
uaccaauuuaugccuacagccuccgc

SEQ ID NO: 154 - RNA, 21 nt, Artificial sequence
  HBV RNAi Agent antisense strand unmodified sequence
uaccaauuuaugccuacaguu

SEQ ID NO: 155 - RNA, 21 nt, Artificial sequence
  HBV RNAi Agent antisense strand unmodified sequence
auugagagaaguccaccacga

SEQ ID NO: 156 - RNA, 21 nt, Artificial sequence
  HBV RNAi Agent antisense strand unmodified sequence
auugagagaaguccaccacuu

SEQ ID NO: 157 - RNA, 21 nt, Artificial sequence
  HBV RNAi Agent antisense strand unmodified sequence
uuugagagaaguccaccacga

SEQ ID NO: 158 - RNA, 21 nt, Artificial sequence
  HBV RNAi Agent antisense strand unmodified sequence
aauugagagaaguccaccacg

SEQ ID NO: 159 - RNA, 21 nt, Artificial sequence
  HBV RNAi Agent antisense strand unmodified sequence
aauugagagaaguccaccauu

SEQ ID NO: 160 - RNA, 21 nt, Artificial sequence
  HBV RNAi Agent antisense strand unmodified sequence
uauugagagaaguccaccacg

SEQ ID NO: 161 - RNA, 21 nt, Artificial sequence
  HBV RNAi Agent antisense strand unmodified sequence
uaccaauuuaugccuacaggu

SEQ ID NO: 162 - RNA, 21 nt, Artificial sequence
  HBV RNAi Agent antisense strand unmodified sequence
uaccaauuuaugccuacagcc

SEQ ID NO: 163 - RNA, 23 nt, Artificial sequence
  HBV RNAi Agent antisense strand unmodified sequence
uaccaauuuaugccuacagccuu

SEQ ID NO: 164 - RNA, 23 nt, Artificial sequence
  HBV RNAi Agent antisense strand unmodified sequence
uaccaauuuaugccuacagccuc

SEQ ID NO: 165 - RNA, 21 nt, Artificial sequence
  HBV RNAi Agent antisense strand unmodified sequence
uuugagagaaguccaccacuu

SEQ ID NO: 166 - RNA, 23 nt, Artificial sequence
  HBV RNAi Agent antisense strand unmodified sequence
auugagagaaguccaccacgguu

SEQ ID NO: 167 - RNA, 23 nt, Artificial sequence
  HBV RNAi Agent antisense strand unmodified sequence
auugagagaaguccaccacgagu

SEQ ID NO: 168 - RNA, 23 nt, Artificial sequence
  HBV RNAi Agent antisense strand unmodified sequence
uauugagagaaguccaccacguu

SEQ ID NO: 169 - RNA, 23 nt, Artificial sequence
  HBV RNAi Agent antisense strand unmodified sequence
uauugagagaaguccaccacgag

SEQ ID NO: 170 - RNA, 22 nt, Artificial sequence
  HBV RNAi Agent antisense strand unmodified sequence
uauugagagaaguccaccacga

SEQ ID NO: 171 - RNA, 21 nt, Artificial sequence
  HBV RNAi Agent antisense strand unmodified sequence
agaaaauugagagaaguccac

SEQ ID NO: 172 - RNA, 22 nt, Artificial sequence
  HBV RNAi Agent antisense strand unmodified sequence
uaccaauuuaugccuacagcuu

SEQ ID NO: 173 - RNA, 22 nt, Artificial sequence
  HBV RNAi Agent antisense strand unmodified sequence
uaccaauuuaugccuacagccu

SEQ ID NO: 174 - RNA, 21 nt, Artificial sequence
  HBV RNAi Agent antisense strand unmodified sequence
uauugagagaaguccaccauu

SEQ ID NO: 175 - RNA, 22 nt, Artificial sequence
  HBV RNAi Agent antisense strand unmodified sequence
uauugagagaaguccaccacuu

SEQ ID NO: 176 - RNA, 22 nt, Artificial sequence
  HBV RNAi Agent antisense strand unmodified sequence
uuugagagaaguccaccacguu

SEQ ID NO: 177 - RNA, 22 nt, Artificial sequence
  HBV RNAi Agent antisense strand unmodified sequence
uuugagagaaguccaccacgag

SEQ ID NO: 178 - RNA, 21 nt, Artificial sequence
  HBV RNAi Agent antisense strand unmodified sequence
agaaaauugagagaaguccuu

SEQ ID NO: 179 - RNA, 23 nt, Artificial sequence
  HBV RNAi Agent antisense strand unmodified sequence
agaaaauugagagaaguccacuu

SEQ ID NO: 180 - RNA, 22 nt, Artificial sequence
  HBV RNAi Agent antisense strand unmodified sequence
agaaaauugagagaaguccacc

SEQ ID NO: 181 - RNA, 21 nt, Artificial sequence
  HBV RNAi Agent antisense strand unmodified sequence
ugaaaauugagagaaguccac

SEQ ID NO: 182 - RNA, 21 nt, Artificial sequence
  HBV RNAi Agent antisense strand unmodified sequence
accaauuuaugccuacagcuu

SEQ ID NO: 183 - RNA, 22 nt, Artificial sequence
  HBV RNAi Agent antisense strand unmodified sequence
accaauuuaugccuacagccuu

SEQ ID NO: 184 - RNA, 22 nt, Artificial sequence
  HBV RNAi Agent antisense strand unmodified sequence
accaauuuaugccuacagccuc

SEQ ID NO: 185 - RNA, 21 nt, Artificial sequence
  HBV RNAi Agent antisense strand unmodified sequence
uccaauuuaugccuacagcuu

SEQ ID NO: 186 - RNA, 22 nt, Artificial sequence
  HBV RNAi Agent antisense strand unmodified sequence
uccaauuuaugccuacagccuu

SEQ ID NO: 187 - RNA, 21 nt, Artificial sequence
  HBV RNAi Agent antisense strand unmodified sequence
uaccaauuuaugccuacagcu

SEQ ID NO: 188 - RNA, 21 nt, Artificial sequence
  HBV RNAi Agent antisense strand unmodified sequence
uaccaauuuaugccuacagcg

SEQ ID NO: 189 - RNA, 21 nt, Artificial sequence
  HBV RNAi Agent antisense strand unmodified sequence
aaccaauuuaugccuacagcc

SEQ ID NO: 190 - RNA, 21 nt, Artificial sequence
  HBV RNAi Agent antisense strand unmodified sequence
accaauuuaugccuacagccu

SEQ ID NO: 191 - RNA, 21 nt, Artificial sequence
  HBV RNAi Agent antisense strand unmodified sequence
uccaauuuaugccuacagccu

SEQ ID NO: 192 - RNA, 21 nt, Artificial sequence
  HBV RNAi Agent antisense strand unmodified sequence
accaauuuaugccuacagccg

SEQ ID NO: 193 - RNA, 21 nt, Artificial sequence
  HBV RNAi Agent antisense strand unmodified sequence
uccaauuuaugccuacagccg

SEQ ID NO: 194 - RNA, 21 nt, Artificial sequence
  HBV RNAi Agent antisense strand unmodified sequence
uaccaauuuaugccuacaggg

SEQ ID NO: 195 - DNA, 25 bp, Artificial sequence
  HBV RNAi Agent sense strand modified sequence
uugccuguaggcauaaauugguaut

SEQ ID NO: 196 - RNA, 26 nt, Artificial sequence
  HBV RNAi Agent sense strand modified sequence
uauaugccuguaggcauaaauuggua

SEQ ID NO: 197 - DNA, 26 bp, Artificial sequence
  HBV RNAi Agent sense strand modified sequence
gcggaggcuguaggcauaaauuggta

SEQ ID NO: 198 - RNA, 21 nt, Artificial sequence
  HBV RNAi Agent sense strand modified sequence
cuguaggcauaaauugguauu

SEQ ID NO: 199 - RNA, 21 nt, Artificial sequence
  HBV RNAi Agent sense strand modified sequence
gccuguaggcauaaauuggua

SEQ ID NO: 200 - RNA, 21 nt, Artificial sequence
  HBV RNAi Agent sense strand modified sequence
gccuguaggcauaaauuggua

SEQ ID NO: 201 - RNA, 21 nt, Artificial sequence
  HBV RNAi Agent sense strand modified sequence
gccuguaggcauaaauuggua

SEQ ID NO: 202 - DNA, 21 bp, Artificial sequence
  HBV RNAi Agent sense strand modified sequence
gccuguaggcauaaauuggta

SEQ ID NO: 203 - RNA, 21 nt, Artificial sequence
  HBV RNAi Agent sense strand modified sequence
aacuguaggcauaaauuggua

SEQ ID NO: 204 - RNA, 21 nt, Artificial sequence
  HBV RNAi Agent sense strand modified sequence
ucgugguggacuucucucaau

SEQ ID NO: 205 - RNA, 21 nt, Artificial sequence
  HBV RNAi Agent sense strand modified sequence
aagugguggacuucucucaau

SEQ ID NO: 206 - DNA, 21 bp, Artificial sequence
  HBV RNAi Agent sense strand modified sequence
ucgugguggacuucucucaat

SEQ ID NO: 207 - RNA, 21 nt, Artificial sequence
  HBV RNAi Agent sense strand modified sequence
cgugguggacuucucucaauu

SEQ ID NO: 208 - RNA, 21 nt, Artificial sequence
  HBV RNAi Agent sense strand modified sequence
aaugguggacuucucucaauu

SEQ ID NO: 209 - DNA, 21 bp, Artificial sequence
  HBV RNAi Agent sense strand modified sequence
cgugguggacuucucucaatt

SEQ ID NO: 210 - RNA, 21 nt, Artificial sequence
  HBV RNAi Agent sense strand modified sequence
ggacuucucucaauuuucuaa

SEQ ID NO: 211 - RNA, 21 nt, Artificial sequence
  HBV RNAi Agent sense strand modified sequence
cgugguggacuucucucaaua

SEQ ID NO: 212 - RNA, 21 nt, Artificial sequence
  HBV RNAi Agent sense strand modified sequence
ucgugguggacuucucucaaa

SEQ ID NO: 213 - RNA, 21 nt, Artificial sequence
  HBV RNAi Agent sense strand modified sequence
accuguaggcauaaauuggua

SEQ ID NO: 214 - RNA, 19 nt, Artificial sequence
  HBV RNAi Agent sense strand modified sequence
cuguaggcauaaauuggua

SEQ ID NO: 215 - RNA, 19 nt, Artificial sequence
  HBV RNAi Agent sense strand modified sequence
cuguaggcauaaauuggua

SEQ ID NO: 216 - RNA, 19 nt, Artificial sequence
  HBV RNAi Agent sense strand modified sequence
cuguaggcauaaauuggua

SEQ ID NO: 217 - RNA, 20 nt, Artificial sequence
  HBV RNAi Agent sense strand modified sequence
acuguaggcauaaauuggua

SEQ ID NO: 218 - RNA, 21 nt, Artificial sequence
  HBV RNAi Agent sense strand modified sequence
ggcuguaggcauaaauuggua

SEQ ID NO: 219 - RNA, 21 nt, Artificial sequence
  HBV RNAi Agent sense strand modified sequence
aagugguggacuucucucaau

SEQ ID NO: 220 - RNA, 21 nt, Artificial sequence
  HBV RNAi Agent sense strand modified sequence
aagugguggacuucucucaaa

SEQ ID NO: 221 - RNA, 21 nt, Artificial sequence
  HBV RNAi Agent sense strand modified sequence
ccgugguggacuucucucaau

SEQ ID NO: 222 - RNA, 21 nt, Artificial sequence
  HBV RNAi Agent sense strand modified sequence
ccgugguggacuucucucaau

SEQ ID NO: 223 - RNA, 22 nt, Artificial sequence
  HBV RNAi Agent sense strand modified sequence
cucgugguggacuucucucaau

SEQ ID NO: 224 - RNA, 19 nt, Artificial sequence
  HBV RNAi Agent sense strand modified sequence
gugguggacuucucucaau

SEQ ID NO: 225 - RNA, 21 nt, Artificial sequence
  HBV RNAi Agent sense strand modified sequence
gugguggacuucucucaauuu

SEQ ID NO: 226 - RNA, 22 nt, Artificial sequence
  HBV RNAi Agent sense strand modified sequence
ucgugguggacuucucucaauu

SEQ ID NO: 227 - RNA, 19 nt, Artificial sequence
  HBV RNAi Agent sense strand modified sequence
ugguggacuucucucaauu

SEQ ID NO: 228 - RNA, 19 nt, Artificial sequence
  HBV RNAi Agent sense strand modified sequence
ugguggacuucucucaauu

SEQ ID NO: 229 - RNA, 21 nt, Artificial sequence
  HBV RNAi Agent sense strand modified sequence
guggacuucucucaauuuucu

SEQ ID NO: 230 - RNA, 21 nt, Artificial sequence
  HBV RNAi Agent sense strand modified sequence
cuguaggcauaaauugguauu

SEQ ID NO: 231 - RNA, 22 nt, Artificial sequence
  HBV RNAi Agent sense strand modified sequence
gcuguaggcauaaauugguauu

SEQ ID NO: 232 - RNA, 23 nt, Artificial sequence
  HBV RNAi Agent sense strand modified sequence
ggcuguaggcauaaauugguauu

SEQ ID NO: 233 - RNA, 23 nt, Artificial sequence
  HBV RNAi Agent sense strand modified sequence
aacuguaggcauaaauugguauu

SEQ ID NO: 234 - RNA, 21 nt, Artificial sequence
  HBV RNAi Agent sense strand modified sequence
ugguggacuucucucaauauu

SEQ ID NO: 235 - RNA, 22 nt, Artificial sequence
  HBV RNAi Agent sense strand modified sequence
gugguggacuucucucaauauu

SEQ ID NO: 236 - RNA, 23 nt, Artificial sequence
  HBV RNAi Agent sense strand modified sequence
aaugguggacuucucucaauauu

SEQ ID NO: 237 - RNA, 23 nt, Artificial sequence
  HBV RNAi Agent sense strand modified sequence
cgugguggacuucucucaauauu

SEQ ID NO: 238 - RNA, 21 nt, Artificial sequence
  HBV RNAi Agent sense strand modified sequence
cgugguggacuucucucaaua

SEQ ID NO: 239 - RNA, 21 nt, Artificial sequence
  HBV RNAi Agent sense strand modified sequence
aagugguggacuucucucaau

SEQ ID NO: 240 - RNA, 21 nt, Artificial sequence
  HBV RNAi Agent sense strand modified sequence
gugguggacuucucucaaauu

SEQ ID NO: 241 - RNA, 22 nt, Artificial sequence
  HBV RNAi Agent sense strand modified sequence
cgugguggacuucucucaaauu

SEQ ID NO: 242 - RNA, 23 nt, Artificial sequence
  HBV RNAi Agent sense strand modified sequence
aagugguggacuucucucaaauu

SEQ ID NO: 243 - RNA, 23 nt, Artificial sequence
  HBV RNAi Agent sense strand modified sequence
ucgugguggacuucucucaaauu

SEQ ID NO: 244 - RNA, 22 nt, Artificial sequence
  HBV RNAi Agent sense strand modified sequence
gugguggacuucucucaauauu

SEQ ID NO: 245 - RNA, 23 nt, Artificial sequence
  HBV RNAi Agent sense strand modified sequence
cgugguggacuucucucaauauu

SEQ ID NO: 246 - RNA, 23 nt, Artificial sequence
  HBV RNAi Agent sense strand modified sequence
cucgugguggacuucucucaaua

SEQ ID NO: 247 - RNA, 25 nt, Artificial sequence
  HBV RNAi Agent sense strand modified sequence
cucgugguggacuucucucaauauu

SEQ ID NO: 248 - RNA, 21 nt, Artificial sequence
  HBV RNAi Agent sense strand modified sequence
ggcuguaggcauaaauuggua

SEQ ID NO: 249 - RNA, 23 nt, Artificial sequence
  HBV RNAi Agent sense strand modified sequence
gaggcuguaggcauaaauuggua

SEQ ID NO: 250 - RNA, 25 nt, Artificial sequence
  HBV RNAi Agent sense strand modified sequence
gaggcuguaggcauaaauugguauu

SEQ ID NO: 251 - RNA, 19 nt, Artificial sequence
  HBV RNAi Agent sense strand modified sequence
ggacuucucucaauuuucu

SEQ ID NO: 252 - RNA, 21 nt, Artificial sequence
  HBV RNAi Agent sense strand modified sequence
guggacuucucucaauuuucu

SEQ ID NO: 253 - RNA, 22 nt, Artificial sequence
  HBV RNAi Agent sense strand modified sequence
gguggacuucucucaauuuucu

SEQ ID NO: 254 - RNA, 19 nt, Artificial sequence
  HBV RNAi Agent sense strand modified sequence
ggacuucucucaauuuuca

SEQ ID NO: 255 - RNA, 19 nt, Artificial sequence
  HBV RNAi Agent sense strand modified sequence
ggacuucucucaauuuuca

SEQ ID NO: 256 - RNA, 19 nt, Artificial sequence
  HBV RNAi Agent sense strand modified sequence
gcuguaggcauaaauuggu

SEQ ID NO: 257 - RNA, 20 nt, Artificial sequence
  HBV RNAi Agent sense strand modified sequence
ggcuguaggcauaaauuggu

SEQ ID NO: 258 - RNA, 22 nt, Artificial sequence
  HBV RNAi Agent sense strand modified sequence
gaggcuguaggcauaaauuggu

SEQ ID NO: 259 - RNA, 19 nt, Artificial sequence
  HBV RNAi Agent sense strand modified sequence
gcuguaggcauaaauugga

SEQ ID NO: 260 - RNA, 20 nt, Artificial sequence
  HBV RNAi Agent sense strand modified sequence
ggcuguaggcauaaauugga

SEQ ID NO: 261 - RNA, 21 nt, Artificial sequence
  HBV RNAi Agent sense strand modified sequence
agcuguaggcauaaauuggua

SEQ ID NO: 262 - RNA, 21 nt, Artificial sequence
  HBV RNAi Agent sense strand modified sequence
cgcuguaggcauaaauuggua

SEQ ID NO: 263 - RNA, 21 nt, Artificial sequence
  HBV RNAi Agent sense strand modified sequence
ggcuguaggcauaaauugguu

SEQ ID NO: 264 - RNA, 21 nt, Artificial sequence
  HBV RNAi Agent sense strand modified sequence
cuguaggcauaaauugguauu

SEQ ID NO: 265 - RNA, 21 nt, Artificial sequence
  HBV RNAi Agent sense strand modified sequence
cuguaggcauaaauugguauu

SEQ ID NO: 266 - RNA, 21 nt, Artificial sequence
  HBV RNAi Agent sense strand modified sequence
aggcuguaggcauaaauuggu

SEQ ID NO: 267 - RNA, 21 nt, Artificial sequence
  HBV RNAi Agent sense strand modified sequence
aggcuguaggcauaaauugga

SEQ ID NO: 268 - RNA, 21 nt, Artificial sequence
  HBV RNAi Agent sense strand modified sequence
cggcuguaggcauaaauuggu

SEQ ID NO: 269 - RNA, 21 nt, Artificial sequence
  HBV RNAi Agent sense strand modified sequence
cggcuguaggcauaaauugga

SEQ ID NO: 270 - RNA, 21 nt, Artificial sequence
  HBV RNAi Agent sense strand modified sequence
cccuguaggcauaaauuggua

SEQ ID NO: 271 - RNA, 21 nt, Artificial sequence
  HBV RNAi Agent sense strand modified sequence
cgcuguaggcauaaauuggua

SEQ ID NO: 272 - RNA, 21 nt, Artificial sequence
  HBV RNAi Agent sense strand modified sequence
cccuguaggcauaaauuggua

SEQ ID NO: 273 - RNA, 21 nt, Artificial sequence
  HBV RNAi Agent sense strand modified sequence
guggacuucucucaauuuucu

SEQ ID NO: 274 - RNA, 21 nt, Artificial sequence
  HBV RNAi Agent sense strand modified sequence
cgcuguaggcauaaauuggua

SEQ ID NO: 275 - DNA, 25 bp, Artificial sequence
  HBV RNAi Agent sense strand unmodified sequence
uugccuguaggcauaaauugguaut

SEQ ID NO: 276 - RNA, 26 nt, Artificial sequence
  HBV RNAi Agent sense strand unmodified sequence
uauaugccuguaggcauaaauuggua

SEQ ID NO: 277 - DNA, 26 bp, Artificial sequence
  HBV RNAi Agent sense strand unmodified sequence
gcggaggcuguaggcauaaauuggta

SEQ ID NO: 278 - RNA, 21 nt, Artificial sequence
  HBV RNAi Agent sense strand unmodified sequence
cuguaggcauaaauugguauu

SEQ ID NO: 279 - RNA, 21 nt, Artificial sequence
  HBV RNAi Agent sense strand unmodified sequence
gccuguaggcauaaauuggua

SEQ ID NO: 280 - DNA, 21 bp, Artificial sequence
  HBV RNAi Agent sense strand unmodified sequence
gccuguaggcauaaauuggta

SEQ ID NO: 281 - RNA, 21 nt, Artificial sequence
  HBV RNAi Agent sense strand unmodified sequence
aacuguaggcauaaauuggua

SEQ ID NO: 282 - RNA, 21 nt, Artificial sequence
  HBV RNAi Agent sense strand unmodified sequence
ucgugguggacuucucucaau

SEQ ID NO: 283 - RNA, 21 nt, Artificial sequence
  HBV RNAi Agent sense strand unmodified sequence
aagugguggacuucucucaau

SEQ ID NO: 284 - DNA, 21 bp, Artificial sequence
  HBV RNAi Agent sense strand unmodified sequence
ucgugguggacuucucucaat

SEQ ID NO: 285 - RNA, 21 nt, Artificial sequence
  HBV RNAi Agent sense strand unmodified sequence
cgugguggacuucucucaauu

SEQ ID NO: 286 - RNA, 21 nt, Artificial sequence
  HBV RNAi Agent sense strand unmodified sequence
aaugguggacuucucucaauu

SEQ ID NO: 287 - DNA, 21 bp, Artificial sequence
  HBV RNAi Agent sense strand unmodified sequence
cgugguggacuucucucaatt

SEQ ID NO: 288 - RNA, 21 nt, Artificial sequence
  HBV RNAi Agent sense strand unmodified sequence
ggacuucucucaauuuucuaa

SEQ ID NO: 289 - RNA, 21 nt, Artificial sequence
  HBV RNAi Agent sense strand unmodified sequence
cgugguggacuucucucaaua

SEQ ID NO: 290 - RNA, 21 nt, Artificial sequence
  HBV RNAi Agent sense strand unmodified sequence
ucgugguggacuucucucaaa

SEQ ID NO: 291 - RNA, 21 nt, Artificial sequence
  HBV RNAi Agent sense strand unmodified sequence
accuguaggcauaaauuggua

SEQ ID NO: 292 - RNA, 19 nt, Artificial sequence
  HBV RNAi Agent sense strand unmodified sequence
cuguaggcauaaauuggua

SEQ ID NO: 293 - RNA, 20 nt, Artificial sequence
  HBV RNAi Agent sense strand unmodified sequence
acuguaggcauaaauuggua

SEQ ID NO: 294 - RNA, 21 nt, Artificial sequence
  HBV RNAi Agent sense strand unmodified sequence
ggcuguaggcauaaauuggua

SEQ ID NO: 295 - RNA, 21 nt, Artificial sequence
  HBV RNAi Agent sense strand unmodified sequence
aagugguggacuucucucaaa

SEQ ID NO: 296 - RNA, 21 nt, Artificial sequence
  HBV RNAi Agent sense strand unmodified sequence
ccgugguggacuucucucaau

SEQ ID NO: 297 - RNA, 22 nt, Artificial sequence
  HBV RNAi Agent sense strand unmodified sequence
cucgugguggacuucucucaau

SEQ ID NO: 298 - RNA, 19 nt, Artificial sequence
  HBV RNAi Agent sense strand unmodified sequence
gugguggacuucucucaau

SEQ ID NO: 299 - RNA, 21 nt, Artificial sequence
  HBV RNAi Agent sense strand unmodified sequence
gugguggacuucucucaauuu

SEQ ID NO: 300 - RNA, 22 nt, Artificial sequence
  HBV RNAi Agent sense strand unmodified sequence
ucgugguggacuucucucaauu

SEQ ID NO: 301 - RNA, 19 nt, Artificial sequence
  HBV RNAi Agent sense strand unmodified sequence
ugguggacuucucucaauu

SEQ ID NO: 302 - RNA, 21 nt, Artificial sequence
  HBV RNAi Agent sense strand unmodified sequence
guggacuucucucaauuuucu

SEQ ID NO: 303 - RNA, 22 nt, Artificial sequence
  HBV RNAi Agent sense strand unmodified sequence
gcuguaggcauaaauugguauu

SEQ ID NO: 304 - RNA, 23 nt, Artificial sequence
  HBV RNAi Agent sense strand unmodified sequence
ggcuguaggcauaaauugguauu

SEQ ID NO: 305 - RNA, 23 nt, Artificial sequence
  HBV RNAi Agent sense strand unmodified sequence
aacuguaggcauaaauugguauu

SEQ ID NO: 306 - RNA, 21 nt, Artificial sequence
  HBV RNAi Agent sense strand unmodified sequence
ugguggacuucucucaauauu

SEQ ID NO: 307 - RNA, 22 nt, Artificial sequence
  HBV RNAi Agent sense strand unmodified sequence
gugguggacuucucucaauauu

SEQ ID NO: 308 - RNA, 23 nt, Artificial sequence
  HBV RNAi Agent sense strand unmodified sequence
aaugguggacuucucucaauauu

SEQ ID NO: 309 - RNA, 23 nt, Artificial sequence
  HBV RNAi Agent sense strand unmodified sequence
cgugguggacuucucucaauauu

SEQ ID NO: 310 - RNA, 21 nt, Artificial sequence
  HBV RNAi Agent sense strand unmodified sequence
gugguggacuucucucaaauu

SEQ ID NO: 311 - RNA, 22 nt, Artificial sequence
  HBV RNAi Agent sense strand unmodified sequence
cgugguggacuucucucaaauu

SEQ ID NO: 312 - RNA, 23 nt, Artificial sequence
  HBV RNAi Agent sense strand unmodified sequence
aagugguggacuucucucaaauu

SEQ ID NO: 313 - RNA, 23 nt, Artificial sequence
  HBV RNAi Agent sense strand unmodified sequence
ucgugguggacuucucucaaauu

SEQ ID NO: 314 - RNA, 23 nt, Artificial sequence
  HBV RNAi Agent sense strand unmodified sequence
cucgugguggacuucucucaaua

SEQ ID NO: 315 - RNA, 25 nt, Artificial sequence
  HBV RNAi Agent sense strand unmodified sequence
cucgugguggacuucucucaauauu

SEQ ID NO: 316 - RNA, 23 nt, Artificial sequence
  HBV RNAi Agent sense strand unmodified sequence
gaggcuguaggcauaaauuggua

SEQ ID NO: 317 - RNA, 25 nt, Artificial sequence
  HBV RNAi Agent sense strand unmodified sequence
gaggcuguaggcauaaauugguauu

SEQ ID NO: 318 - RNA, 19 nt, Artificial sequence
  HBV RNAi Agent sense strand unmodified sequence
ggacuucucucaauuuucu

SEQ ID NO: 319 - RNA, 22 nt, Artificial sequence
  HBV RNAi Agent sense strand unmodified sequence
gguggacuucucucaauuuucu

SEQ ID NO: 320 - RNA, 19 nt, Artificial sequence
  HBV RNAi Agent sense strand unmodified sequence
ggacuucucucaauuuuca

SEQ ID NO: 321 - RNA, 21 nt, Artificial sequence
  HBV RNAi Agent sense strand unmodified sequence
guggacuucucucaauuuuca

SEQ ID NO: 322 - RNA, 19 nt, Artificial sequence
  HBV RNAi Agent sense strand unmodified sequence
gcuguaggcauaaauuggu

SEQ ID NO: 323 - RNA, 20 nt, Artificial sequence
  HBV RNAi Agent sense strand unmodified sequence
ggcuguaggcauaaauuggu

SEQ ID NO: 324 - RNA, 22 nt, Artificial sequence
  HBV RNAi Agent sense strand unmodified sequence
gaggcuguaggcauaaauuggu

SEQ ID NO: 325 - RNA, 19 nt, Artificial sequence
  HBV RNAi Agent sense strand unmodified sequence
gcuguaggcauaaauugga

SEQ ID NO: 326 - RNA, 20 nt, Artificial sequence
  HBV RNAi Agent sense strand unmodified sequence
ggcuguaggcauaaauugga

SEQ ID NO: 327 - RNA, 21 nt, Artificial sequence
  HBV RNAi Agent sense strand unmodified sequence
agcuguaggcauaaauuggua

SEQ ID NO: 328 - RNA, 21 nt, Artificial sequence
  HBV RNAi Agent sense strand unmodified sequence
cgcuguaggcauaaauuggua

SEQ ID NO: 329 - RNA, 21 nt, Artificial sequence
  HBV RNAi Agent sense strand unmodified sequence
ggcuguaggcauaaauugguu

SEQ ID NO: 330 - RNA, 21 nt, Artificial sequence
  HBV RNAi Agent sense strand unmodified sequence
aggcuguaggcauaaauuggu

SEQ ID NO: 331 - RNA, 21 nt, Artificial sequence
  HBV RNAi Agent sense strand unmodified sequence
aggcuguaggcauaaauugga

SEQ ID NO: 332 - RNA, 21 nt, Artificial sequence
  HBV RNAi Agent sense strand unmodified sequence
cggcuguaggcauaaauuggu

SEQ ID NO: 333 - RNA, 21 nt, Artificial sequence
  HBV RNAi Agent sense strand unmodified sequence
cggcuguaggcauaaauugga

SEQ ID NO: 334 - RNA, 21 nt, Artificial sequence
  HBV RNAi Agent sense strand unmodified sequence
cccuguaggcauaaauuggua